European Patent Application EP 4 194 019 A1, published June 14, 2023. Title: Method for manufacturing high-functional bioengineered organs using aptamer. Applicant: SNU R&DB FOUNDATION. The sequence listing filed with the application follows.

SEQUENCE LISTING (41 sequences)

SEQ ID NO: 1 - DNA, 40 bp, Artificial Sequence
  anti-CD31 aptamer, wherein n is NapdU [5-(N-Napthylcarboxyamide)-2'-deoxyuridine]
gnagaggaggnacgnaangncngggnanaccccganaann

SEQ ID NO: 2 - DNA, 22 bp, Artificial Sequence
  human GAPDH_F
tgatgacatcaagaaggtggtg

SEQ ID NO: 3 - DNA, 21 bp, Artificial Sequence
  human GAPDH_R
accctgttgctgtagccaaat

SEQ ID NO: 4 - DNA, 21 bp, Artificial Sequence
  human ITGB1_F
cgtagcaaaggaacagcagag

SEQ ID NO: 5 - DNA, 25 bp, Artificial Sequence
  human ITGB1_R
ggtagtagaggtcaatgggatagtc

SEQ ID NO: 6 - DNA, 20 bp, Artificial Sequence
  human ITGB3_F
cctcatcaccatccacgacc

SEQ ID NO: 7 - DNA, 21 bp, Artificial Sequence
  human ITGB3_R
gttgttggctgtgtcccattt

SEQ ID NO: 8 - DNA, 22 bp, Artificial Sequence
  human VE-cadherin_F
cttcacccagaccaagtacaca

SEQ ID NO: 9 - DNA, 20 bp, Artificial Sequence
  human VE-cadherin_R
aatggtgaaagcgtcctggt

SEQ ID NO: 10 - DNA, 20 bp, Artificial Sequence
  human CLDN5_F
aagtgtacgactcggtgctg

SEQ ID NO: 11 - DNA, 20 bp, Artificial Sequence
  human CLDN5_R
aaacaggtagagcacgcctc

SEQ ID NO: 12 - DNA, 23 bp, Artificial Sequence
  human NOS3_F
aaagacaaggcagcagtggaaat

SEQ ID NO: 13 - DNA, 22 bp, Artificial Sequence
  human NOS3_R
tccacgatggtgactttggcta

SEQ ID NO: 14 - DNA, 18 bp, Artificial Sequence
  human CD63_F
cagctagagagccccgga

SEQ ID NO: 15 - DNA, 20 bp, Artificial Sequence
  human CD63_R
ttcattcctccttccaccgc

SEQ ID NO: 16 - DNA, 24 bp, Artificial Sequence
  human PLSCR1_F
ggcagccagagaactgttttaatc

SEQ ID NO: 17 - DNA, 20 bp, Artificial Sequence
  human PLSCR1_R
ggcaagtttgtttccgggtg

SEQ ID NO: 18 - DNA, 17 bp, Artificial Sequence
  human TBXAS1_F
tgcagagcacggttccc

SEQ ID NO: 19 - DNA, 22 bp, Artificial Sequence
  human TBXAS1_R
gtggagtaccatttcaggaggg

SEQ ID NO: 20 - DNA, 20 bp, Artificial Sequence
  human THBS1_F
agtcgtctctgcaacaaccc

SEQ ID NO: 21 - DNA, 22 bp, Artificial Sequence
  human THBS1_R
acaggcatccatcaattggaca

SEQ ID NO: 22 - DNA, 21 bp, Artificial Sequence
  human ALB_F
cgctattagttcgttacacca

SEQ ID NO: 23 - DNA, 20 bp, Artificial Sequence
  human ALB_R
tttacaacatttgctgccca

SEQ ID NO: 24 - DNA, 20 bp, Artificial Sequence
  human CYP1A2_F
cggacagcacttccctgaga

SEQ ID NO: 25 - DNA, 20 bp, Artificial Sequence
  human CYP1A2_R
aggcaggtagcgaaggatgg

SEQ ID NO: 26 - DNA, 20 bp, Artificial Sequence
  rat Gapdh_F
accacagtccatgccatcac

SEQ ID NO: 27 - DNA, 20 bp, Artificial Sequence
  rat Gapdh_R
tccaccaccctgttgctgta

SEQ ID NO: 28 - DNA, 19 bp, Artificial Sequence
  rat Cd63_F
catcaagaagcgtcgggga

SEQ ID NO: 29 - DNA, 20 bp, Artificial Sequence
  rat Cd63_R
acctgaactgctacgccaat

SEQ ID NO: 30 - DNA, 20 bp, Artificial Sequence
  rat Plscr1_F
ctgcgaggctttagggagag

SEQ ID NO: 31 - DNA, 20 bp, Artificial Sequence
  rat Plscr1_R
ctctgaggtctgcaaggtgg

SEQ ID NO: 32 - DNA, 20 bp, Artificial Sequence
  rat Thbs1_F
tagctggaaatgtggtgcgt

SEQ ID NO: 33 - DNA, 20 bp, Artificial Sequence
  rat Thbs1_R
agcaagcatcaggcacttct

SEQ ID NO: 34 - DNA, 20 bp, Artificial Sequence
  rat alpha-Sma_F
catcaccaactgggacgaca

SEQ ID NO: 35 - DNA, 20 bp, Artificial Sequence
  rat alpha-Sma_R
tccgttagcaaggtcggatg

SEQ ID NO: 36 - DNA, 20 bp, Artificial Sequence
  rat Vimentin_F
cactcacctgcgaagtggat

SEQ ID NO: 37 - DNA, 20 bp, Artificial Sequence
  rat Vimentin_R
tggtattcacgaaggtggcg

SEQ ID NO: 38 - DNA, 20 bp, Artificial Sequence
  rat Tgf-beta1_F
ctgctgacccccactgatac

SEQ ID NO: 39 - DNA, 20 bp, Artificial Sequence
  rat Tgf-beta1_R
agccctgtattccgtctcct

SEQ ID NO: 40 - DNA, 20 bp, Artificial Sequence
  rat Timp1_F
tgctcaaaggattcgacgct

SEQ ID NO: 41 - DNA, 20 bp, Artificial Sequence
  rat Timp1_R
agcagggctcagattatgcc